European Patent Application EP 4 710 948 A1, published March 18, 2026. Title: A RECOMBINANT SARS-COV-2 S GLYCOPROTEIN TRIMER, PROTEOLIPOSOMES COMPRISING SUCH A TRIMER AND THEIR USE AS A VACCINE. Applicant: UNIVERSITE GRENOBLE ALPES. The sequence listing filed with the application follows.

SEQUENCE LISTING (15 sequences)

SEQ ID NO: 1 - protein, 1063 aa, synthetic construct
MFVFLVLLPLVSSQCVNLTTRTQLPPAYTNSFTRGVYYPDKVFRSSVLHSTQDLFLPFFSNVTWFHAIHVSGTNGTKRFDNPVLPFNDGVYFASTEKSNIIRGWIFGTTLDSKTQSLLIVNNATNVVIKVCEFQFCNDPFLGVYYHKNNKSWMESEFRVYSSANNCTFEYVSQPFLMDLEGKQGNFKNLREFVFKNIDGYFKIYSKHTPINLVRDLPQGFSALEPLVDLPIGINITRFQTLLALHRSYLTPGDSSSGWTAGAAAYYVGYLQPRTFLLKYNENGTITDAVDCALDPLSETKCTLKSFTVEKGIYQTSNFRVQPTESIVRFPNGSGSGSSTNLVKNKCVNFNFNGLTGTGVLTESNKKFLPFQQFGRDIADTTDAVRDPQTLEILDITPCSFGGVSVITPGTNTSNQVAVLYQDVNCTEVPVAIHADQLTPTWRVYSTGSNVFQTRAGCLIGAEHVNNSYECDIPIGAGICASYQTQTNSPGSASSVASQSIIAYTMSLGAENSVAYSNNSIAIPTNFTISVTTEILPVSMTKTSVDCTMYICGDSTECSNLLLQYGSFCTQLNRALTGIAVEQDKNTQEVFAQVKQIYKTPPIKDFGGFNFSQILPDPSKPSKRSPIEDLLFNKVTLADAGFIKQYGDCLGDIAARDLICAQKFNGLTVLPPLLTDEMIAQYTSALLAGTITSGWTFGAGPALQIPFPMQMAYRFNGIGVTQNVLYENQKLIANQFNSAIGKIQDSLSSTPSALGKLQDVVNQNAQALNTLVKQLSSNFGAISSVLNDILSRLDPPEAEVQIDRLITGRLQSLQTYVTQQLIRAAEIRASANLAATKMSECVLGQSKRVDFCGKGYHLMSFPQSAPHGVVFLHVTYVPAQEKNFTTAPAICHDGKAHFPREGVFVSNGTHWFVTQRNFYEPQIITTDNTFVSGNCDVVIGIVNNTVYDPLQPELDSFKEELDKYFKNHTSPDVDLGDISGINASVVNIQKEIDRLNEVAKNLNESLIDLQELGKYEQGSGYIPEAPRDGQAYVRKDGEWVLLSTFLGRSGSGHHHHHHHHGSGC

SEQ ID NO: 2 - DNA, 3210 bp, synthetic construct
  source 1..3210: mol_type = other DNA
ggtaccgccaccatgttcgtgttcctggtgctcctgcctctggtgagcagccagtgcgtgaacctgaccacccgaacccagctcccaccagcctacaccaacagctttacacggggcgtgtactaccctgacaaggtgttcagatctagcgtcctgcacagcactcaggacctcttcctgccgttcttcagcaacgtgacatggttccacgccatccacgtgagcggcacaaacggaaccaagcggtttgataaccccgtcctgccattcaatgatggagtttacttcgccagtaccgagaagagtaacatcatccggggctggatcttcggcaccaccctggatagcaaaacacagagcctcctgatcgtgaacaatgccacgaacgtcgtgatcaaggtgtgcgagttccagttttgcaatgatcctttcctgggtgtgtactaccacaagaacaacaagagctggatggaaagcgagttcagagtctacagcagcgccaacaactgcacattcgagtacgtctctcagccttttctgatggaccttgaggggaaacaaggcaacttcaagaacctgagagaattcgtgttcaagaacatcgacggctacttcaaaatctactccaagcacacacccatcaacctggtccgggacctccctcagggcttcagcgccctggaacccctggtcgacctgcccataggcatcaacataacgcggttccaaaccctgctggccctgcatagatcctacctgactcctggcgacagcagcagcggatggaccgccggagctgcagcctactatgtgggctacctgcaacctagaaccttcctgctgaagtacaacgagaacggcacaatcacagacgccgtcgactgcgccctggaccctctctctgagacaaagtgcaccctgaagtccttcaccgtggaaaagggcatctaccagaccagcaacttccgggtgcagcctacagagagcatcgtgcgatttccaaacggcagcggcagcggcagctccaccaatctggttaagaacaaatgcgtgaacttcaacttcaacggcctgaccgggaccggcgtgctgaccgaaagcaacaaaaagttcctccccttccagcagttcggccgtgatatcgctgacaccacagatgccgtcagagatccacagaccctggaaatcctggatattacaccctgctccttcggaggagtttctgtgatcacccccgggaccaataccagcaaccaggtggctgtgctgtaccaagatgttaactgcaccgaggttcctgtggccatccacgccgatcagctgacacctacttggagagtgtactccactggctccaatgtgttccagaccagggccggatgtctgatcggcgccgagcacgtgaataacagttacgagtgcgacatccctatcggcgccggcatctgtgccagctaccagacccagacaaacagccctgggtctgcttcctctgtagctagccagagcatcatcgcctacaccatgagcctgggcgcagagaacagcgtggcctattccaacaactctatcgccattcccaccaactttacaattagcgtcacaacagagatcctgcccgtgagcatgaccaagaccagcgtggactgtacaatgtacatctgtggcgacagcactgaatgcagcaacctgctgctgcaatacggctccttttgcacccaactgaaccgggcgctgaccggaatcgccgtggaacaggacaaaaatacccaggaggtgttcgcccaagtgaagcagatctacaagaccccacctatcaaggacttcggcggctttaactttagccagattctccctgatccttctaagcctagcaagcggagccctatcgaggatctgctgttcaacaaggtcaccctggccgatgccggctttatcaaacagtatggcgattgcctgggcgacatagccgccagagatctgatctgcgcccagaaattcaacggcctgacagttctcccacctctgctgaccgacgagatgatcgctcagtacacctctgccctgctggctggcaccatcacatctgggtggacatttggcgccggccccgccctgcagatcccctttcccatgcagatggcctatagattcaacggaatcggcgtgacccagaacgtgctgtatgaaaaccagaagctgatcgctaaccagttcaattctgccatcggcaagatccaggactccctctcctctacccccagcgccctgggcaaactgcaggacgtggtgaatcagaacgcccaagccctgaacaccctggtgaagcagctcagcagcaattttggcgccatcagctctgtgctgaacgatatcctgtctagactggaccctccagaagccgaagtccagatcgatagactgatcacaggcagactgcagtccctgcaaacctacgtgacccaacagctgatcagggccgctgaaataagagccagcgccaatctcgccgctaccaagatgtccgagtgtgtgctgggacagtctaaacgcgttgacttctgcggcaaaggctatcacctgatgagcttcccccagagcgcgccgcacggcgtggtgttcctgcatgtgacatacgtgcctgcccaagagaagaatttcacaaccgcccctgccatctgccacgacggcaaggcccacttcccaagagagggcgttttcgtttccaatggcacacactggttcgtgacacaaagaaacttctacgaaccccagattatcaccaccgacaacaccttcgtgagtggcaattgtgacgtggtcatcggaatcgtgaacaacacagtgtacgaccctctgcaacctgagctggactcttttaaggaagagctggacaagtactttaaaaaccacaccagccccgatgtggacctgggcgacatcagtggcattaacgccagcgtggtgaacatccaaaaggaaatcgacagactgaacgaggtggccaagaacctgaacgagtccctgatcgacctgcaggagctcggcaaatacgagcagggatccggatacatccccgaggcccccagagatggccaggcctacgtgcggaaggacggcgagtgggtactgctgagcacattcctgggcagatccggcagcggccatcaccaccatcaccaccatcatggcagcggctgctgactcgag

SEQ ID NO: 3 - protein, 4 aa, synthetic construct
GSAS

SEQ ID NO: 4 - protein, 30 aa, synthetic construct
GYIPEAPRDGQAYVRKDGEWVLLSTFLGRS

SEQ ID NO: 5 - protein, 15 aa, synthetic construct
GSGHHHHHHHHGSGC

SEQ ID NO: 6 - DNA, 20 bp, synthetic construct
  source 1..20: mol_type = other DNA
ctggtcaaggttaatatagg

SEQ ID NO: 7 - DNA, 19 bp, synthetic construct
  source 1..19: mol_type = other DNA
ggtaactggtatgatttcg

SEQ ID NO: 8 - DNA, 19 bp, synthetic construct
  source 1..19: mol_type = other DNA
  misc_feature <1: product = FLUOROPHORE FAM
  misc_feature >19: product = BHQ1 quencher
tcatacaaaccacgccagg

SEQ ID NO: 9 - DNA, 23 bp, synthetic construct
  source 1..23: mol_type = other DNA
cgatctcttgtagatctgttctc

SEQ ID NO: 10 - DNA, 22 bp, synthetic construct
  source 1..22: mol_type = other DNA
atattgcagcagtacgcacaca

SEQ ID NO: 11 - DNA, 26 bp, synthetic construct
  source 1..26: mol_type = other DNA
  misc_feature <1: product = HEXACHLOROFLUORESCEIN
  misc_feature >26: product = BHQ1 quencher
acactagccatccttactgcgcttcg

SEQ ID NO: 12 - protein, 6 aa, synthetic construct
GSGSGS

SEQ ID NO: 13 - protein, 11 aa, synthetic construct
GSGHHHHHHHH

SEQ ID NO: 14 - protein, 12 aa, synthetic construct
GSGHHHHHHHHK

SEQ ID NO: 15 - protein, 16 aa, synthetic construct
GSGHHHHHHHHKGRGR